European Patent Application EP 4 163 298 A1, published April 12, 2023. Title: GRP94 specific antibody or antigen-binding fragment thereof and uses thereof. Applicant: Kookmin University Industry Academy Cooperation Foundation. The sequence listing filed with the application follows.

SEQUENCE LISTING (67 sequences)

SEQ ID NO: 1 - protein, 10 aa, Artificial Sequence
  Amino acid sequence of HCDR1 of GRP94 B5
GFTFSNYYMS

SEQ ID NO: 2 - protein, 17 aa, Artificial Sequence
  Amino acid sequence of HCDR2 of GRP94 B5
GIYPNSGSTYYADSVKG

SEQ ID NO: 3 - protein, 12 aa, Artificial Sequence
  Amino acid sequence of HCDR3 of GRP94 B5
DPLHPARFPFDY

SEQ ID NO: 4 - protein, 13 aa, Artificial Sequence
  Amino acid sequence of LCDR1 of GRP94 B5
TGSSSNIGNNAVS

SEQ ID NO: 5 - protein, 7 aa, Artificial Sequence
  Amino acid sequence of LCDR2 of GRP94 B5
ADSHRPS

SEQ ID NO: 6 - protein, 9 aa, Artificial Sequence
  Amino acid sequence of LCDR3 of GRP94 B5
GAWDASLNA

SEQ ID NO: 7 - protein, 121 aa, Artificial Sequence
  Amino acid sequence of heavy chain variable of GRP94 B5
EVQLLESGGGLVQPGGSLRLSCAASGFTFSNYYMSWVRQAPGKGLEWVSGIYPNSGSTYYADSVKGRFTISRDNSKNTLYLQMNSLRAEDTAVYYCARDPLHPARFPFDYWGQGTLVTVSS

SEQ ID NO: 8 - protein, 110 aa, Artificial Sequence
  Amino acid sequence of light chain variable of GRP94 B5
QSVLTQPPSASGTPGQRVTISCTGSSSNIGNNAVSWYQQLPGTAPKLLIYADSHRPSGVPDRFSGSKSGTSASLAISGLRSEDEADYYCGAWDASLNAYVFGGGTKLTVL

SEQ ID NO: 9 - protein, 10 aa, Artificial Sequence
  Amino acid sequence of HCDR1 of GRP94 E5
GFTFSNYAMS

SEQ ID NO: 10 - protein, 17 aa, Artificial Sequence
  Amino acid sequence of HCDR2 of GRP94 E5
GISSSSGSTYYADSVKG

SEQ ID NO: 11 - protein, 12 aa, Artificial Sequence
  Amino acid sequence of HCDR3 of GRP94 E5
DRHPFSPNWFDY

SEQ ID NO: 12 - protein, 13 aa, Artificial Sequence
  Amino acid sequence of LCDR1 of GRP94 E5
SGSPSNIGSNTVT

SEQ ID NO: 13 - protein, 7 aa, Artificial Sequence
  Amino acid sequence of LCDR2 of GRP94 E5
ADSHRPS

SEQ ID NO: 14 - protein, 9 aa, Artificial Sequence
  Amino acid sequence of LCDR3 of GRP94 E5
ASWDDSLNG

SEQ ID NO: 15 - protein, 121 aa, Artificial Sequence
  Amino acid sequence of heavy chain variable of GRP94 E5
EVQLLESGGGLVQPGGSLRLSCAASGFTFSNYAMSWVRQAPGKGLEWVSGISSSSGSTYYADSVKGRFTTSRDNSKNTLYLQMNSLRAEDTAVYYCARDRHPFSPNWFDYWGQGTLVTVSS

SEQ ID NO: 16 - protein, 110 aa, Artificial Sequence
  Amino acid sequence of light chain variable of GRP94 E5
QSVLTQPPSASGTPGQRVTISCSGSPSNIGSNTVTWYQQLPGTAPKLLIYADSHRPSGVPDRFSGSKSGTSASLAISGLRSEDEADYYCASWDDSLNGYVFGGGTKLTVL

SEQ ID NO: 17 - protein, 10 aa, Artificial Sequence
  Amino acid sequence of HCDR1 of GRP94 2H5
GFTFSGYAMS

SEQ ID NO: 18 - protein, 17 aa, Artificial Sequence
  Amino acid sequence of HCDR2 of GRP94 2H5
AISHGGSSKYYADSVKG

SEQ ID NO: 19 - protein, 18 aa, Artificial Sequence
  Amino acid sequence of HCDR3 of GRP94 2H5
DLLSPLQSIGSYDDAMDV

SEQ ID NO: 20 - protein, 13 aa, Artificial Sequence
  Amino acid sequence of LCDR1 of GRP94 2H5
SGSSSNIGSNTVS

SEQ ID NO: 21 - protein, 7 aa, Artificial Sequence
  Amino acid sequence of LCDR2 of GRP94 2H5
ADNNRPS

SEQ ID NO: 22 - protein, 9 aa, Artificial Sequence
  Amino acid sequence of LCDR3 of GRP94 2H5
ASWDDSLNA

SEQ ID NO: 23 - protein, 127 aa, Artificial Sequence
  Amino acid sequence of heavy chain variable of GRP94 2H5
EVQLLESGGGLVQPGGSLRLSCAASGFTFSGYAMSWVRQAPGKGLEWVSAISHGGSSKYYADSVKGRFTISRDNSKNTLYLQMNSLRAEDTAVYYCAKDLLSPLQSIGSYDDAMDVWGQGTLVTVSS

SEQ ID NO: 24 - protein, 110 aa, Artificial Sequence
  Amino acid sequence of light chain variable of GRP94 2H5
QSVLTQPPSASGTPGQRVTISCSGSSSNIGSNTVSWYQQLPGTAPKLLIYADNNRPSGVPDRFSGSKSGTSASLAISGLRSEDEADYYCASWDDSLNAYVFGGGTKLTVL

SEQ ID NO: 25 - protein, 10 aa, Artificial Sequence
  Amino acid sequence of HCDR1 of GRP94 3G7
GFTFSNYSMS

SEQ ID NO: 26 - protein, 17 aa, Artificial Sequence
  Amino acid sequence of HCDR2 of GRP94 3G7
GIYYGSGNKYYADSVKG

SEQ ID NO: 27 - protein, 7 aa, Artificial Sequence
  Amino acid sequence of HCDR3 of GRP94 3G7
NLASFDY

SEQ ID NO: 28 - protein, 13 aa, Artificial Sequence
  Amino acid sequence of LCDR1 of GRP94 3G7
SGSSSNIGSNSVN

SEQ ID NO: 29 - protein, 7 aa, Artificial Sequence
  Amino acid sequence of LCDR2 of GRP94 3G7
SNSHRPS

SEQ ID NO: 30 - protein, 9 aa, Artificial Sequence
  Amino acid sequence of LCDR3 of GRP94 3G7
GTWDSSLSG

SEQ ID NO: 31 - protein, 116 aa, Artificial Sequence
  Amino acid sequence of heavy chain variable of GRP94 3G7
EVQLLESGGGLVQPGGSLRLSCAASGFTFSNYSMSWVRQAPGKGLEWVSGIYYGSGNKYYADSVKGRFTISRDNSKNTLYLQMNSLRAEDTAVYYCAKNLASFDYWGQGTLVTVSS

SEQ ID NO: 32 - protein, 110 aa, Artificial Sequence
  Amino acid sequence of light chain variable of GRP94 3G7
QSVLTQPPSASGTPGQRVTISCSGSSSNIGSNSVNWYQQLPGTAPKLLIYSNSHRPSGVPDRFSGSKSGTSASLAISGLRSEDEADYYCGTWDSSLSGYVFGGGTKLTVL

SEQ ID NO: 33 - DNA, 30 bp, Artificial Sequence
  Nucleic acid sequence of HCDR1 of GRP94 B5
ggattcacctttagcaattattatatgagc

SEQ ID NO: 34 - DNA, 51 bp, Artificial Sequence
  Nucleic acid sequence of HCDR2 of GRP94 B5
gggatctatcctaatagtggtagtacatattacgctgattctgtaaaaggt

SEQ ID NO: 35 - DNA, 36 bp, Artificial Sequence
  Nucleic acid sequence of HCDR3 of GRP94 B5
gatcctcttcatccggcgcgttttccgttcgactac

SEQ ID NO: 36 - DNA, 39 bp, Artificial Sequence
  Nucleic acid sequence of LCDR1 of GRP94 B5
actggctcttcatctaatattggcaataatgctgtctcc

SEQ ID NO: 37 - DNA, 21 bp, Artificial Sequence
  Nucleic acid sequence of LCDR2 of GRP94 B5
gctgatagtcatcggccaagc

SEQ ID NO: 38 - DNA, 27 bp, Artificial Sequence
  Nucleic acid sequence of LCDR3 of GRP94 B5
ggtgcttgggatgctagcctgaatgct

SEQ ID NO: 39 - DNA, 363 bp, Artificial Sequence
  Nucleic acid sequence of heavy chain variable of GRP94 B5
gaggtgcagctgttggagtctgggggaggcttggtacagcctggggggtccctgagactctcctgtgcagcctctggattcacctttagcaattattatatgagctgggtccgccaggctccagggaaggggctggagtgggtctcagggatctatcctaatagtggtagtacatattacgctgattctgtaaaaggtcggttcaccatctccagagacaattccaagaacacgctgtatctgcaaatgaacagcctgagagccgaggacacggccgtgtattactgtgcgagagatcctcttcatccggcgcgttttccgttcgactactggggccagggtacactggtcaccgtgagctca

SEQ ID NO: 40 - DNA, 330 bp, Artificial Sequence
  Nucleic acid sequence of light chain variable of GRP94 B5
cagtctgtgctgactcagccaccctcagcgtctgggacccccgggcagagggtcaccatctcttgtactggctcttcatctaatattggcaataatgctgtctcctggtaccagcagctcccaggaacggcccccaaactcctcatctatgctgatagtcatcggccaagcggggtccctgaccgattctctggctccaagtctggcacctcagcctccctggccatcagtgggctccggtccgaggatgaggctgattattactgtggtgcttgggatgctagcctgaatgcttatgtcttcggcggaggcaccaagctgacggtccta

SEQ ID NO: 41 - DNA, 30 bp, Artificial Sequence
  Nucleic acid sequence of HCDR1 of GRP94 E5
ggattcacctttagcaattatgctatgagc

SEQ ID NO: 42 - DNA, 51 bp, Artificial Sequence
  Nucleic acid sequence of HCDR2 of GRP94 E5
gggatctcttctagtagtggtagtacatattacgctgattctgtaaaaggt

SEQ ID NO: 43 - DNA, 36 bp, Artificial Sequence
  Nucleic acid sequence of HCDR3 of GRP94 E5
gatcgtcatccgttttcgcctaattggttcgactac

SEQ ID NO: 44 - DNA, 39 bp, Artificial Sequence
  Nucleic acid sequence of LCDR1 of GRP94 E5
agtggctctccatctaatattggcagtaatactgtcacc

SEQ ID NO: 45 - DNA, 21 bp, Artificial Sequence
  Nucleic acid sequence of LCDR2 of GRP94 E5
gctgatagtcatcggccaagc

SEQ ID NO: 46 - DNA, 27 bp, Artificial Sequence
  Nucleic acid sequence of LCDR3 of GRP94 E5
gcttcttgggatgatagcctgaatggt

SEQ ID NO: 47 - DNA, 363 bp, Artificial Sequence
  Nucleic acid sequence of heavy chain variable of GRP94 E5
gaggtgcagctgttggagtctgggggaggcttggtacagcctggggggtccctgagactctcctgtgcggcctctggattcacctttagcaattatgctatgagctgggtccgccaggctccagggaaggggctggagtgggtctcagggatctcttctagtagtggtagtacatattacgctgattctgtaaaaggtcggttcaccacctccagagacaattccaagaacacgctgtatctgcaaatgaacagcctgagagccgaggacacggccgtgtattactgtgcgagagatcgtcatccgttttcgcctaattggttcgactactggggccagggtacactggtcaccgtgagctca

SEQ ID NO: 48 - DNA, 330 bp, Artificial Sequence
  Nucleic acid sequence of light chain variable of GRP94 E5
cagtctgtgctgactcagccaccctcagcgtctgggacccccgggcagagggtcaccatctcttgtagtggctctccatctaatattggcagtaatactgtcacctggtaccagcagctcccaggaacggcccccaaactcctcatctatgctgatagtcatcggccaagcggggtccctgaccgattctctggctccaagtctggcacctcagcctccctggccatcagtgggctccggtccgaggatgaggctgattattactgtgcttcttgggatgatagcctgaatggttatgtcttcggcggaggcaccaagctgacggtccta

SEQ ID NO: 49 - DNA, 30 bp, Artificial Sequence
  Nucleic acid sequence of HCDR1 of GRP94 2H5
ggattcacctttagcggttatgctatgagc

SEQ ID NO: 50 - DNA, 51 bp, Artificial Sequence
  Nucleic acid sequence of HCDR2 of GRP94 2H5
gcgatctctcatggtggtagtagtaaatattacgctgattctgtaaaaggt

SEQ ID NO: 51 - DNA, 54 bp, Artificial Sequence
  Nucleic acid sequence of HCDR3 of GRP94 2H5
gatcttcttagtcctctgcagagtattgggtcttatgatgatgctatggacgtc

SEQ ID NO: 52 - DNA, 39 bp, Artificial Sequence
  Nucleic acid sequence of LCDR1 of GRP94 2H5
agtggctcttcatctaatattggcagtaatactgtctcc

SEQ ID NO: 53 - DNA, 21 bp, Artificial Sequence
  Nucleic acid sequence of LCDR2 of GRP94 2H5
gctgataataatcggccaagc

SEQ ID NO: 54 - DNA, 27 bp, Artificial Sequence
  Nucleic acid sequence of LCDR3 of GRP94 2H5
gcttcttgggatgatagcctgaatgct

SEQ ID NO: 55 - DNA, 381 bp, Artificial Sequence
  Nucleic acid sequence of heavy chain variable of GRP94 2H5
gaggtgcagctgttggagtctgggggaggcttggtacagcctggggggtccctgagactctcctgtgcagcctctggattcacctttagcggttatgctatgagctgggtccgccaggctccagggaaggggctggagtgggtctcagcgatctctcatggtggtagtagtaaatattacgctgattctgtaaaaggtcggttcaccatctccagagacaattccaagaacacgctgtatctgcaaatgaacagcctgagagccgaggacacggccgtgtattactgtgcgaaagatcttcttagtcctctgcagagtattgggtcttatgatgatgctatggacgtctggggccagggtacactggtcaccgtgagctca

SEQ ID NO: 56 - DNA, 330 bp, Artificial Sequence
  Nucleic acid sequence of light chain variable of GRP94 2H5
cagtctgtgctgactcagccaccctcagcgtctgggacccccgggcagagggtcaccatctcttgtagtggctcttcatctaatattggcagtaatactgtctcctggtaccagcagctcccaggaacggcccccaaactcctcatctatgctgataataatcggccaagcggggtccctgaccgattctctggctccaagtctggcacctcagcctccctggccatcagtgggctccggtccgaggatgaggctgattattactgtgcttcttgggatgatagcctgaatgcttatgtcttcggcgggggcaccaagctgacggtccta

SEQ ID NO: 57 - DNA, 30 bp, Artificial Sequence
  Nucleic acid sequence of HCDR1 of GRP94 3G7
ggattcacctttagcaattattctatgagc

SEQ ID NO: 58 - DNA, 51 bp, Artificial Sequence
  Nucleic acid sequence of HCDR2 of GRP94 3G7
gggatctattatggtagtggtaataaatattacgctgattctgtaaaaggt

SEQ ID NO: 59 - DNA, 21 bp, Artificial Sequence
  Nucleic acid sequence of HCDR3 of GRP94 3G7
aatctggcttcgttcgactac

SEQ ID NO: 60 - DNA, 39 bp, Artificial Sequence
  Nucleic acid sequence of LCDR1 of GRP94 3G7
agtggctcttcatctaatattggcagtaattctgtcaac

SEQ ID NO: 61 - DNA, 21 bp, Artificial Sequence
  Nucleic acid sequence of LCDR2 of GRP94 3G7
tctaatagtcatcggccaagc

SEQ ID NO: 62 - DNA, 27 bp, Artificial Sequence
  Nucleic acid sequence of LCDR3 of GRP94 3G7
ggtacttgggattctagcctgagtggt

SEQ ID NO: 63 - DNA, 348 bp, Artificial Sequence
  Nucleic acid sequence of heavy chain variable of GRP94 3G7
gaggtgcagctgttggagtctgggggaggcttggtacagcctggggggtccctgagactctcctgtgcagcctctggattcacctttagcaattattctatgagctgggtccgccaggctccagggaaggggctggagtgggtctcagggatctattatggtagtggtaataaatattacgctgattctgtaaaaggtcggttcaccatctccagagacaattccaagaacacgctgtatctgcaaatgaacagcctgagagccgaggacacggccgtgtattactgtgcgaaaaatctggcttcgttcgactactggggccagggtacactggtcaccgtgagctca

SEQ ID NO: 64 - DNA, 330 bp, Artificial Sequence
  Nucleic acid sequence of light chain variable of GRP94 3G7
cagtctgtgctgactcagccaccctcagcgtctgggacccccgggcagagggtcaccatctcttgtagtggctcttcatctaatattggcagtaattctgtcaactggtaccagcagctcccaggaacggcccccaaactcctcatctattctaatagtcatcggccaagcggggtccctgaccgattctctggctccaagtctggcacctcagcctccctggccatcagtgggctccggtccgaggacgaggctgattattactgtggtacttgggattctagcctgagtggttatgtcttcggcggaggcaccaagctgacggtccta

SEQ ID NO: 65 - protein, 803 aa, Artificial Sequence
  Wilt-type rhGRP94
MRALWVLGLCCVLLTFGSVRADDEVDVDGTVEEDLGKSREGSRTDDEVVQREEEAIQLDGLNASQIRELREKSEKFAFQAEVNRMMKLIINSLYKNKEIFLRELISNASDALDKIRLISLTDENALSGNEELTVKIKCDKEKNLLHVTDTGVGMTREELVKNLGTIAKSGTSEFLNKMTEAQEDGQSTSELIGQFGVGFYSAFLVADKVIVTSKHNNDTQHIWESDSNEFSVIADPRGNTLGRGTTITLVLKEEASDYLELDTIKNLVKKYSQFINFPIYVWSSKTETVEEPMEEEEAAKEEKEESDDEAAVEEEEEEKKPKTKKVEKTVWDWELMNDIKPIWQRPSKEVEEDEYKAFYKSFSKESDDPMAYIHFTAEGEVTFKSILFVPTSAPRGLFDEYGSKKSDYIKLYVRRVFITDDFHDMMPKYLNFVKGVVDSDDLPLNVSRETLQQHKLLKVIRKKLVRKTLDMIKKIADDKYNDTFWKEFGTNIKLGVIEDHSNRTRLAKLLRFQSSHHPTDITSLDQYVERMKEKQDKIYFMAGSSRKEAESSPFVERLLKKGYEVIYLTEPVDEYCIQALPEFDGKRFQNVAKEGVKFDESEKTKESREAVEKEFEPLLNWMKDKALKDKIEKAVVSQRLTESPCALVASQYGWSGNMERIMKAQAYQTGKDISTNYYASQKKTFEINPRHPLIRDMLRRIKEDEDDKTVLDLAVVLFETATLRSGYLLPDTKAYGDRIERMLRLSLNIDPDAKVEEEPEEEPEETAEDTTEDTEQDEDEEMDVGTDEEEETAKESTAEKDEL

SEQ ID NO: 66 - protein, 777 aa, Artificial Sequence
  rhGRP94 Part. 1 (Asp 22- Glu 799)
DDEVDVDGTVEEDLGKSREGSRTDDEVVQREEEAIQLDGLNASQIRELREKSEKFAFQAEVNRMMKLIINSLYKNKEIFLRELISNASDALDKIRLISLTDENALSGNEELTVKIKCDKEKNLLHVTDTGVGMTREELVKNLGTIAKSGTSEFLNKMTEAQEDGQSTSELIGQFGVGFYSAFLVADKVIVTSKHNNDTQHIWESDSNEFSVIADPRGNTLGRGTTITLVLKEEASDYLELDTIKNLVKKYSQFINFPIYVWSSKTETVEEPMEEEEAAKEEKEESDDEAAVEEEEEEKKPKTKKVEKTVWDWELMNDIKPIWQRPSKEVEEDEYKAFYKSFSKESDDPMAYIHFTAEGEVTFKSILFVPTSAPRGLFDEYGSKKSDYIKLYVRRVFITDDFHDMMPKYLNFVKGVVDSDDLPLNVSRETLQQHKLLKVIRKKLVRKTLDMIKKIADDKYNDTFWKEFGTNIKLGVIEDHSNRTRLAKLLRFQSSHHPTDITSLDQYVERMKEKQDKIYFMAGSSRKEAESSPFVERLLKKGYEVIYLTEPVDEYCIQALPEFDGKRFQNVAKEGVKFDESEKTKESREAVEKEFEPLLNWMKDKALKDKIEKAVVSQRLTESPCALVASQYGWSGNMERIMKAQAYQTGKDISTNYYASQKKTFEINPRHPLIRDMLRRIKEDEDDKTVLDLAVVLFETATLRSGYLLPDTKAYGDRIERMLRLSLNIDPDAKVEEEPEEEPEETAEDTTEDTEQDEDEEMDVGTDEEETAKESTAE

SEQ ID NO: 67 - protein, 198 aa, Artificial Sequence
  rhGRP94 part. 4 (Glu 602 - Glu 799)
EKTKESREAVEKEFEPLLNWMKDKALKDKIEKAVVSQRLTESPCALVASQYGWSGNMERIMKAQAYQTGKDISTNYYASQKKTFEINPRHPLIRDMLRRIKEDEDDKTVLDLAVVLFETATLRSGYLLPDTKAYGDRIERMLRLSLNIDPDAKVEEEPEEEPEETAEDTTEDTEQDEDEEMDVGTDEEEETAKESTAE